European Patent Specification EP 3 808 774 B1, published April 16, 2025. Title: HUMAN IL-4R BINDING ANTIBODY, ANTIGEN BINDING FRAGMENT THEREOF, AND MEDICAL USE THEREOF. Applicant: JIANGSU HENGRUI MEDICINE CO., LTD.; SHANGHAI HENGRUI PHARMACEUTICAL CO., LTD. The sequence listing filed with the application follows.

SEQUENCE LISTING (46 sequences)

SEQ ID NO: 1 - protein, 118 aa, Artificial Sequence
  DOMAIN (1)..(118): murine mAb 25G7 heavy chain variable region
EVQLVESGGGLVKPGGSLKLSCAASGFTFSDYGMHWVRQAPEKGLEWVAFISSGSSIIYYADIVKGRSTISRDNAKNTLFLQMTSLRSEDTAMYYCTRGNKRGFFDYWGQGTILTVSS

SEQ ID NO: 2 - protein, 108 aa, Artificial Sequence
  DOMAIN (1)..(108): murine mAb 25G7 light chain variable region
QIVLTQSPALMSASPGEKVTMTCNASSSVSYMYWYQRKPRSSPKPWIYLTSNLASGVPVRFSGSGSGTSYSLTISSMEAEDAATYYCQQWRSNPPMLTFGSGTKLEVK

SEQ ID NO: 3 - protein, 10 aa, Artificial Sequence
  DOMAIN (1)..(10): murine mAb 25G7 HCDR1
GFTFSDYGMH

SEQ ID NO: 4 - protein, 17 aa, Artificial Sequence
  DOMAIN (1)..(17): murine mAb 25G7 HCDR2
FISSGSSIIYYADIVKG

SEQ ID NO: 5 - protein, 9 aa, Artificial Sequence
  DOMAIN (1)..(9): murine mAb 25G7 HCDR3
GNKRGFFDY

SEQ ID NO: 6 - protein, 10 aa, Artificial Sequence
  DOMAIN (1)..(10): murine mAb 25G7 LCDR1
NASSSVSYMY

SEQ ID NO: 7 - protein, 7 aa, Artificial Sequence
  DOMAIN (1)..(7): murine mAb 25G7 LCDR2
LTSNLAS

SEQ ID NO: 8 - protein, 11 aa, Artificial Sequence
  DOMAIN (1)..(11): murine mAb 25G7 LCDR3
QQWRSNPPMLT

SEQ ID NO: 9 - protein, 125 aa, Artificial Sequence
  DOMAIN (1)..(125): murine mAb 7B10 heavy chain variable region
QVQLQQPGTELLKPGASVSLSCKASGYTFTSYWMHWVKQRPGQGLEWIGLIHPNSDTTKFSENFKTRATLTIDKSSSTAYMKLSSLTSEDSAVYYCAKSKIITTIVARHWYFDVWGTGTTVTVSS

SEQ ID NO: 10 - protein, 111 aa, Artificial Sequence
  DOMAIN (1)..(111): murine mAb 7B10 light chain variable region
DIVLTQSPPSLAVSLGQRATISCKASQSVDYGGDSYMNWYQQKLGQPPKVLIYAASNLESGIPARFSGSGSGTDFTLNIHPVEEEDVATYYCQHSNENPPTFGGGTKLEIK

SEQ ID NO: 11 - protein, 10 aa, Artificial Sequence
  DOMAIN (1)..(10): murine mAb 7B10 HCDR1
GYTFTSYWMH

SEQ ID NO: 12 - protein, 17 aa, Artificial Sequence
  DOMAIN (1)..(17): murine mAb 7B10 HCDR2
LIHPNSDTTKFSENFKT

SEQ ID NO: 13 - protein, 16 aa, Artificial Sequence
  DOMAIN (1)..(16): murine mAb 7B10 HCDR3
SKIITTIVARHWYFDV

SEQ ID NO: 14 - protein, 15 aa, Artificial Sequence
  DOMAIN (1)..(14): murine mAb 7B10 LCDR1
KASQSVDYGGDSYMN

SEQ ID NO: 15 - protein, 7 aa, Artificial Sequence
  DOMAIN (1)..(7): murine mAb 7B10 LCDR2
AASNLES

SEQ ID NO: 16 - protein, 9 aa, Artificial Sequence
  DOMAIN (1)..(9): murine mAb 7B10 LCDR3
QHSNENPPT

SEQ ID NO: 17 - protein, 445 aa, Artificial Sequence
  CHAIN (1)..(445): humanized antibody hu25G7 heavy chain
EVQLVESGGGLVQPGGSLRLSCAASGFTFSDYGMHWVRQAPGKGLEWVAFISSGSSIIYYADIVKGRSTISRDNAKNSLYLQMNSLRAEDTAVYYCTRGNKRGFFDYWGQGTLVTVSSASTKGPSVFPLAPCSRSTSESTAALGCLVKDYFPEPVTVSWNSGALTSGVHTFPAVLQSSGLYSLSSVVTVPSSSLGTKTYTCNVDHKPSNTKVDKRVESKYGPPCPPCPAPEFLGGPSVFLFPPKPKDTLMISRTPEVTCVVVDVSQEDPEVQFNWYVDGVEVHNAKTKPREEQFNSTYRVVSVLTVLHQDWLNGKEYKCKVSNKGLPSSIEKTISKAKGQPREPQVYTLPPSQEEMTKNQVSLTCLVKGFYPSDIAVEWESNGQPENNYKTTPPVLDSDGSFFLYSRLTVDKSRWQEGNVFSCSVMHEALHNHYTQKSLSLSLGK

SEQ ID NO: 18 - protein, 215 aa, Artificial Sequence
  CHAIN (1)..(215): humanized antibody hu25G7 light chain
EIVLTQSPATLSLSPGERATLSCNASSSVSYMYWYQQKPGQAPRLLIYLTSNLASGIPARFSGSGSGTDFTLTISSLEPEDFAVYYCQQWRSNPPMLTFGGGTKVEIKRTVAAPSVFIFPPSDEQLKSGTASVVCLLNNFYPREAKVQWKVDNALQSGNSQESVTEQDSKDSTYSLSSTLTLSKADYEKHKVYACEVTHQGLSSPVTKSFNRGEC

SEQ ID NO: 19 - protein, 455 aa, Artificial Sequence
  CHAIN (1)..(455): humanized antibody hu7B10 heavy chain
EVQLVQSGAEVKKPGASVKVSCKASGYTFTSYWMHWVRQAPGQGLEWMGLIHPNSDTTKFSENFKTRVTMTIDTSISTAYMELSRLRSDDTAVYYCAKSKIITTIVARHWYFDVWGQGTTVTVSSASTKGPSVFPLAPSSKSTSGGTAALGCLVKDYFPEPVTVSWNSGALTSGVHTFPAVLQSSGLYSLSSVVTVPSSSLGTQTYICNVNHKPSNTKVDKKVEPKSCDKTHTCPPCPAPELLGGPSVFLFPPKPKDTLMISRTPEVTCVVVDVSHEDPEVKFNWYVDGVEVHNAKTKPREEQYNSTYRVVSVLTVLHQDWLNGKEYKCKVSNKALPAPIEKTISKAKGQPREPQVYTLPPSREEMTKNQVSLTCLVKGFYPSDIAVEWESNGQPENNYKTTPPVLDSDGSFFLYSKLTVDKSRWQQGNVFSCSVMHEALHNHYTQKSLSLSPGK

SEQ ID NO: 20 - protein, 218 aa, Artificial Sequence
  CHAIN (1)..(218): humanized antibody hu7B10 light chain
DIVLTQTPLSLSVTPGQPASISCKASQSVDYGGDSYMNWYLQKPGQPPQLLIYAASNLESGVPDRFSGSGSGTDFTLKISRVEAEDVGVYYCQHSNENPPTFGGGTKVEIKRTVAAPSVFIFPPSDEQLKSGTASVVCLLNNFYPREAKVQWKVDNALQSGNSQESVTEQDSKDSTYSLSSTLTLSKADYEKHKVYACEVTHQGLSSPVTKSFNRGEC

SEQ ID NO: 21 - protein, 98 aa, Artificial Sequence
  DOMAIN (1)..(98): human germline heavy chain template IGHV3-48*01
EVQLVESGGGLVQPGGSLRLSCAASGFTFSSYSMNWVRQAPGKGLEWVSYISSSSSTIYYADSVKGRFTISRDNAKNSLYLQMNSLRAEDTAVYYCAR

SEQ ID NO: 22 - protein, 95 aa, Artificial Sequence
  DOMAIN (1)..(95): human germline light chain template IGKV3-11*01
EIVLTQSPATLSLSPGERATLSCRASQSVSSYLAWYQQKPGQAPRLLIYDASNRATGIPARFSGSGSGTDFTLTISSLEPEDFAVYYCQQRSNWP

SEQ ID NO: 23 - protein, 98 aa, Artificial Sequence
  DOMAIN (1)..(98): human germline heavy chain template IGHV1-2*02
QVQLVQSGAEVKKPGASVKVSCKASGYTFTGYYMHWVRQAPGQGLEWMGWINPNSGGTNYAQKFQGRVTMTRDTSISTAYMELSRLRSDDTAVYYCAR

SEQ ID NO: 24 - protein, 100 aa, Artificial Sequence
  DOMAIN (1)..(100): human germline light chain template IGKV2D-29*01
DIVMTQTPLSLSVTPGQPASISCKSSQSLLHSDGKTYLYWYLQKPGQPPQLLIYEVSNRFSGVPDRFSGSGSGTDFTLKISRVEAEDVGVYYCMQSIQLP

SEQ ID NO: 25 - protein, 118 aa, Artificial Sequence
  DOMAIN (1)..(118): hu25G7-VH-a
EVQLVESGGGLVQPGGSLRLSCAASGFTFSDYGMHWVRQAPGKGLEWVAFISSGSSIIYYADIVKGRFTISRDNAKNSLYLQMNSLRAEDTAVYYCARGNKRGFFDYWGQGTLVTVSS

SEQ ID NO: 26 - protein, 118 aa, Artificial Sequence
  DOMAIN (1)..(118): hu25G7-VH-b
EVQLVESGGGLVQPGGSLRLSCAASGFTFSDYGMHWVRQAPGKGLEWVAFISSGSSIIYYADIVKGRFTISRDNAKNSLYLQMNSLRAEDTAVYYCTRGNKRGFFDYWGQGTLVTVSS

SEQ ID NO: 27 - protein, 118 aa, Artificial Sequence
  DOMAIN (1)..(118): hu25G7-VH-c
EVQLVESGGGLVQPGGSLRLSCAASGFTFSDYGMHWVRQAPGKGLEWVAFISSGSSIIYYADIVKGRSTISRDNAKNSLYLQMNSLRAEDTAVYYCTRGNKRGFFDYWGQGTLVTVSS

SEQ ID NO: 28 - protein, 108 aa, Artificial Sequence
  DOMAIN (1)..(108): hu25G7-VL-a
EIVLTQSPATLSLSPGERATLSCNASSSVSYMYWYQQKPGQAPRLLIYLTSNLASGIPARFSGSGSGTDFTLTISSLEPEDFAVYYCQQWRSNPPMLTFGGGTKVEIK

SEQ ID NO: 29 - protein, 108 aa, Artificial Sequence
  DOMAIN (1)..(108): hu25G7-VL-b
EIVLTQSPATLSLSPGERATLSCNASSSVSYMYWYQQKPGQAPRLLIYLTSNLASGIPARFSGSGSGTDYTLTISSLEPEDFAVYYCQQWRSNPPMLTFGGGTKVEIK

SEQ ID NO: 30 - protein, 108 aa, Artificial Sequence
  DOMAIN (1)..(108): hu25G7-VL-c
EIVLTQSPATLSLSPGERATLSCNASSSVSYMYWYQQKPGQAPRPWIYLTSNLASGIPARFSGSGSGTDYTLTISSLEPEDFAVYYCQQWRSNPPMLTFGGGTKVEIK

SEQ ID NO: 31 - protein, 125 aa, Artificial Sequence
  DOMAIN (1)..(125): hu7B10-VH-a
EVQLVQSGAEVKKPGASVKVSCKASGYTFTSYWMHWVRQAPGQGLEWMGLIHPNSDTTKFSENFKTRVTMTRDTSISTAYMELSRLRSDDTAVYYCARSKIITTIVARHWYFDVWGQGTTVTVSS

SEQ ID NO: 32 - protein, 125 aa, Artificial Sequence
  DOMAIN (1)..(125): hu7B10-VH-b
EVQLVQSGAEVKKPGASVKVSCKASGYTFTSYWMHWVRQAPGQGLEWMGLIHPNSDTTKFSENFKTRVTMTIDTSISTAYMELSRLRSDDTAVYYCAKSKIITTIVARHWYFDVWGQGTTVTVSS

SEQ ID NO: 33 - protein, 125 aa, Artificial Sequence
  DOMAIN (1)..(125): hu7B10-VH-c
EVQLVQSGAEVKKPGASVKVSCKASGYTFTSYWMHWVRQAPGQGLEWMGLIHPNSDTTKFSENFKTRVTLTIDKSISTAYMELSRLRSDDTAVYYCAKSKIITTIVARHWYFDVWGQGTTVTVSS

SEQ ID NO: 34 - protein, 111 aa, Artificial Sequence
  DOMAIN (1)..(111): hu7B10-VL-a
DIVMTQTPLSLSVTPGQPASISCKASQSVDYGGDSYMNWYLQKPGQPPQLLIYAASNLESGVPDRFSGSGSGTDFTLKISRVEAEDVGVYYCQHSNENPPTFGGGTKVEIK

SEQ ID NO: 35 - protein, 111 aa, Artificial Sequence
  DOMAIN (1)..(111): hu7B10-VL-b
DIVLTQTPLSLSVTPGQPASISCKASQSVDYGGDSYMNWYLQKPGQPPQLLIYAASNLESGVPDRFSGSGSGTDFTLKISRVEAEDVGVYYCQHSNENPPTFGGGTKVEIK

SEQ ID NO: 36 - protein, 111 aa, Artificial Sequence
  DOMAIN (1)..(111): hu7B10-VL-c
DIVMTQTPLSLSVTPGQPASISCKASQSVDYGGDSYMNWYLQKPGQPPQLLIYAASNLESGIPDRFSGSGSGTDFTLKISRVEAEDVGVYYCQHSNENPPTFGGGTKVEIK

SEQ ID NO: 37 - protein, 108 aa, Artificial Sequence
  DOMAIN (1)..(108): hu25G7-A light chain variable region
EIVLTQSPATLSLSPGERATLSCRASSSVPYMYWYQQKPGQAPRLLIYLTSNLASGIPARFSGSGSGTDFTLTISSLEPEDFAVYYCQQWRAYPPMLTFGGGTKVEIK

SEQ ID NO: 38 - protein, 10 aa, Artificial Sequence
  DOMAIN (1)..(10): hu25G7-A LCDR1
RASSSVPYMY

SEQ ID NO: 39 - protein, 7 aa, Artificial Sequence
  DOMAIN (1)..(7): hu25G7-B LCDR2
LASSRPS

SEQ ID NO: 40 - protein, 11 aa, Artificial Sequence
  DOMAIN (1)..(11): hu25G7-A LCDR3
QQWRAYPPMLT

SEQ ID NO: 41 - protein, 108 aa, Artificial Sequence
  DOMAIN (1)..(108): hu25G7-B light chain variable region
EIVLTQSPATLSLSPGERATLSCRASPGVPPLAWYQQKPGQAPRLLIYLASSRPSGIPARFSGSGSGTDFTLTISSLEPEDFAVYYCQQWRSNPPMLTFGGGTKVEIK

SEQ ID NO: 42 - protein, 10 aa, Artificial Sequence
  DOMAIN (1)..(10): hu25G7-B LCDR1
RASPGVPPLA

SEQ ID NO: 43 - protein, 118 aa, Artificial Sequence
  DOMAIN (1)..(118): hu25G7-VH-c optimized heavy chain variable region
EVQLVESGGGLVQPGGSLRLSCAASGFTFSDYGMHWVRQAPGKGLEWVAFISSGSSIIYYADIVKGRSTISRDNAKNTLYLQMNSLRAEDTAVYYCTRGNKRGFFDYWGQGTLVTVSS

SEQ ID NO: 44 - protein, 445 aa, Artificial Sequence
  CHAIN (1)..(445): hu25G7-A and hu25G7-B heavy chain
EVQLVESGGGLVQPGGSLRLSCAASGFTFSDYGMHWVRQAPGKGLEWVAFISSGSSIIYYADIVKGRSTISRDNAKNTLYLQMNSLRAEDTAVYYCTRGNKRGFFDYWGQGTLVTVSSASTKGPSVFPLAPCSRSTSESTAALGCLVKDYFPEPVTVSWNSGALTSGVHTFPAVLQSSGLYSLSSVVTVPSSSLGTKTYTCNVDHKPSNTKVDKRVESKYGPPCPPCPAPEFLGGPSVFLFPPKPKDTLMISRTPEVTCVVVDVSQEDPEVQFNWYVDGVEVHNAKTKPREEQFNSTYRVVSVLTVLHQDWLNGKEYKCKVSNKGLPSSIEKTISKAKGQPREPQVYTLPPSQEEMTKNQVSLTCLVKGFYPSDIAVEWESNGQPENNYKTTPPVLDSDGSFFLYSRLTVDKSRWQEGNVFSCSVMHEALHNHYTQKSLSLSLGK

SEQ ID NO: 45 - protein, 215 aa, Artificial Sequence
  CHAIN (1)..(215): hu25G7-A light chain
EIVLTQSPATLSLSPGERATLSCRASSSVPYMYWYQQKPGQAPRLLIYLTSNLASGIPARFSGSGSGTDFTLTISSLEPEDFAVYYCQQWRAYPPMLTFGGGTKVEIKRTVAAPSVFIFPPSDEQLKSGTASVVCLLNNFYPREAKVQWKVDNALQSGNSQESVTEQDSKDSTYSLSSTLTLSKADYEKHKVYACEVTHQGLSSPVTKSFNRGEC

SEQ ID NO: 46 - protein, 215 aa, Artificial Sequence
  CHAIN (1)..(215): hu25G7-B light chain
EIVLTQSPATLSLSPGERATLSCRASPGVPPLAWYQQKPGQAPRLLIYLASSRPSGIPARFSGSGSGTDFTLTISSLEPEDFAVYYCQQWRSNPPMLTFGGGTKVEIKRTVAAPSVFIFPPSDEQLKSGTASVVCLLNNFYPREAKVQWKVDNALQSGNSQESVTEQDSKDSTYSLSSTLTLSKADYEKHKVYACEVTHQGLSSPVTKSFNRGEC